European Patent Application EP 4 253 410 A1, published October 4, 2023. Title: RAS MUTANT EPITOPE PEPTIDE AND T CELL RECEPTOR RECOGNIZING RAS MUTANT. Applicant: SHANGHAI GENBASE BIOTECHNOLOGY CO., LTD. The sequence listing filed with the application follows.

SEQUENCE LISTING (69 sequences)

SEQ ID NO: 1 - protein, 188 aa, Artificial Sequence
  RAS G12V mutant amino acid sequence
MTEYKLVVVGAVGVGKSALTIQLIQNHFVDEYDPTIEDSYRKQVVIDGETCLLDILDTAGQEEYSAMRDQYMRTGEGFLCVFAINNTKSFEDIHHYREQIKRVKDSEDVPMVLVGNKCDLPSRTVDTKQAQDLARSYGIPFIETSAKTRQGVDDAFYTLVREIRKHKEKMSKDGKKKKKKSKTKCVIM

SEQ ID NO: 2 - protein, 11 aa, Artificial Sequence
  RAS G12V mutant amino acid sequence aa3-13/G12V-T9
EYKLVVVGAVG

SEQ ID NO: 3 - protein, 12 aa, Artificial Sequence
  RAS G12V mutant amino acid sequence aa2-13/G12V-T3
TEYKLVVVGAVG

SEQ ID NO: 4 - protein, 12 aa, Artificial Sequence
  RAS G12V mutant amino acid sequence aa3-14/G12V-T16
EYKLVVVGAVGV

SEQ ID NO: 5 - protein, 13 aa, Artificial Sequence
  RAS G12V mutant amino acid sequence aa2-14/G12V-T15
TEYKLVVVGAVGV

SEQ ID NO: 6 - protein, 134 aa, Artificial Sequence
  B13.14.1 TCR V(alpha) amino acid sequence
MASAPISMLAMLFTLSGLRAQSVAQPEDQVNVAEGNPLTVKCTYSVSGNPYLFWYVQYPNRGLQFLLKYITGDNLVKGSYGFEAEFNKSQTSFHLKKPSALVSDSALYFCAVRDGRGGGNKLTFGTGTQLKVEL

SEQ ID NO: 7 - protein, 133 aa, Artificial Sequence
  B13.14.1 TCR V(beta) amino acid sequence
MSNQVLCCVVLCLLGANTVDGGITQSPKYLFRKEGQNVTLSCEQNLNHDAMYWYRQDPGQGLRLIYYSQIVNDFQKGDIAEGYSVSREKKESFPLTVTSAQKNPTAFYLCASSPGQRDNSPLHFGNGTRLTVT

SEQ ID NO: 8 - protein, 6 aa, Artificial Sequence
  B13.14.1 TCR CDR1(alpha) amino acid sequence
VSGNPY

SEQ ID NO: 9 - protein, 8 aa, Artificial Sequence
  B13.14.1 TCR CDR2(alpha) amino acid sequence
YITGDNLV

SEQ ID NO: 10 - protein, 13 aa, Artificial Sequence
  B13.14.1 TCR CDR3(alpha) amino acid sequence
AVRDGRGGGNKLT

SEQ ID NO: 11 - protein, 5 aa, Artificial Sequence
  B13.14.1 TCR CDR1(beta) amino acid sequence
LNHDA

SEQ ID NO: 12 - protein, 6 aa, Artificial Sequence
  B13.14.1 TCR CDR2(beta) amino acid sequence
SQIVND

SEQ ID NO: 13 - protein, 13 aa, Artificial Sequence
  B13.14.1 TCR CDR3(beta) amino acid sequence
ASSPGQRDNSPLH

SEQ ID NO: 14 - DNA, 2012 bp, Artificial Sequence
  Ras G12V-mRNA nucleotide sequence
cttgttctttttgcagaagctcagaataaacgctcaactttgggccaccatgccccggcagctcagcgcggcggccgcgctcttcgcgtccctggccgtaattttgcacgatggcagtcaaatgagagcaaaagcatttccagaaaccagagattattctcaacctactgcagcagcaacagtacaggacataaaaaaacctgtccagcaaccagctaagcaagcacctcaccaaactttagcagcaagattcatggatggtcatatcacctttcaaacagcggccacagtaaaaattccaacaactaccccagcgactacaaaaaacactgcaaccaccagcccaattacctacaccctggtcacaacccaggccacacccaacaactcacacacagctcctccagttactgaagttacagtcggccctagcttagccccttattcactgccacccaccatcaccccaccagctcatacaactggaaccagttcatcaaccgtcagccacacaactgggaacaccactcaacccagtaaccagaccacccttccagcaactttatcgatagcactgcacaaaagcacaaccggtcagaagcctgttcaacccacccatgccccaggaacaacggcagctgcccacaataccacccgcacagctgcacctgcctccacggttcctgggcccacccttgcacctcagccatcgtcagtcaagactggaatttatcaggttctaaacggaagcagactctgtataaaagcagagatggggatacagctgattgttcaagacaaggagtcggttttttcacctcggagatacttcaacatcgaccccaacgcaacgcaagcctctgggaactgtggcacccgaaaatccaaccttctgttgaattttcagggcggatttgtgaatctcacatttaccaaggatgaagaatcatattatatcagtgaagtgggagcctatttgaccgtctcagatccagagacaatttaccaaggaatcaaacatgcggtggtgatgttccagacagcagtcgggcattccttcaagtgcgtgagtgaacagagcctccagttgtcagcccacctgcaggtgaaaacaaccgatgtccaacttcaagcctttgattttgaagatgaccactttggaaatgtggatgagtgctcgtctgactacacaactgaatataaacttgtggtagttggagctgttggcgtaggcaagagtgccttgacgatacagctaattcagaatcattttgtggacgaatatgatccaacaatagaggattcctacaggaagcaagtagtaattgatggagaaacctgtctcttggatattctcgacacagcaggtcaagaggagtacagtgcaatgagggaccagtacatgaggactggggagggctttctttgtgtatttgccataaataatactaaatcatttgaagatattcaccattatagagaacaaattaaaagagttaaggactctgaagatgtacctatggtcctagtaggaaataaatgtgatttgccttctagaacagtagacacaaaacaggctcaggacttagcaagaagttatggaattccttttattgaaacatcagcaaagacaagacagggtgttgatgatgccttctatacattagttcgagaaattcgaaaacataaagaaaagatgagcaaagatggtaaaaagaagaaaaagaagtcaaagacaaagtgtgtaattatgattgtgcttcctgtgattggggccatcgtggttggtctctgccttatgggtatgggtgtctataaaatccgcctaaggtgtcaatcatctggataccagagaatctaatcctctagaggatctggttaccactaaaccagcctcaagaacacccgaatggagtctctaagctacataataccaacttacacttacaaaatgttgtcccccaaaatgtagccattcgtatctgctcctaataaaaagaaagtttcttcac

SEQ ID NO: 15 - DNA, 402 bp, Artificial Sequence
  B13.14.1 TCR V(alpha) nucleotide sequence
atggcctctgcacccatctcgatgcttgcgatgctcttcacattgagtgggctgagagctcagtcagtggctcagccggaagatcaggtcaacgttgctgaagggaatcctctgactgtgaaatgcacctattcagtctctggaaacccttatcttttttggtatgttcaataccccaaccgaggcctccagttccttctgaaatacatcacaggggataacctggttaaaggcagctatggctttgaagctgaatttaacaagagccaaacctccttccacctgaagaaaccatctgcccttgtgagcgactccgctttgtacttctgtgctgtgagagacggtaggggaggaggaaacaaactcacctttgggacaggcactcagctaaaagtggaactc

SEQ ID NO: 16 - DNA, 399 bp, Artificial Sequence
  B13.14.1 TCR V(beta) nucleotide sequence
atgagcaaccaggtgctctgctgtgtggtcctttgtctcctgggagcaaacaccgtggatggtggaatcactcagtccccaaagtacctgttcagaaaggaaggacagaatgtgaccctgagttgtgaacagaatttgaaccacgatgccatgtactggtaccgacaggacccagggcaagggctgagattgatctactactcacagatagtaaatgactttcagaaaggagatatagctgaagggtacagcgtctctcgggagaagaaggaatcctttcctctcactgtgacatcggcccaaaagaacccgacagctttctatctctgtgccagtagccccggacaacgagataattcacccctccactttgggaacgggaccaggctcactgtgaca

SEQ ID NO: 17 - protein, 13 aa, Artificial Sequence
  Ras WT-T15
TEYKLVVVGAGGV

SEQ ID NO: 18 - protein, 137 aa, Artificial Sequence
  Murine TCR(alpha)constant region amino acid sequence
DIQNPEPAVYQLKDPRSQDSTLCLFTDFDSQINVPKTMESGTFITDKTVLDMKAMDSKSNGAIAWSNQTSFTCQDIFKETNATYPSSDVPCDATLTEKSFETDMNLNFQNLSVMGLRILLLKVAGFNLLMTLRLWSS

SEQ ID NO: 19 - DNA, 411 bp, Artificial Sequence
  Murine TCR(alpha)constant region nucleotide sequence
gacatccagaacccagaacctgctgtgtaccagttaaaagatcctcggtctcaggacagcaccctctgcctgttcaccgactttgactcccaaatcaatgtgccgaaaaccatggaatctggaacgttcatcactgacaaaactgtgctggacatgaaagctatggattccaagagcaatggggccattgcctggagcaaccagacaagcttcacctgccaagatatcttcaaagagaccaacgccacctaccccagttcagacgttccctgtgatgccacgttgactgagaaaagctttgaaacagatatgaacctaaactttcaaaacctgtcagttatgggactccgaatcctcctgctgaaagtagccggatttaacctgctcatgacgctgaggctgtggtccagt

SEQ ID NO: 20 - protein, 173 aa, Artificial Sequence
  Murine TCR(beta)constant region amino acid sequence
EDLRNVTPPKVSLFEPSKAEIANKQKATLVCLARGFFPDHVELSWWVNGKEVHSGVSTDPQAYKESNYSYCLSSRLRVSATFWHNPRNHFRCQVQFHGLSEEDKWPEGSPKPVTQNISAEAWGRADCGITSASYQQGVLSATILYEILLGKATLYAVLVSTLVVMAMVKRKNS

SEQ ID NO: 21 - DNA, 519 bp, Artificial Sequence
  Murine TCR(beta)constant region nucleotide sequence
gaggacctgcgcaacgtcaccccaccaaaggtcagtttgtttgagccatcaaaggcggagatcgccaacaaacagaaagctacgctcgtgtgtttggctcggggcttcttcccagaccacgtagaactttcctggtgggtcaatggaaaggaggttcattccggagtgtccactgatccccaagcgtacaaggaatccaactatagctactgtctctcatctcggctccgggtgagtgcgacattctggcataatcctcggaaccactttcgatgccaagtgcagtttcatgggttgagcgaggaagacaagtggcccgagggcagtcctaaaccagtcactcaaaacataagcgccgaggcatggggtagagccgattgtgggattactagcgcttcataccaacaaggggtattgagcgctacaattctttacgaaattctcctcggcaaggcgacgctctacgccgtactggtgtctactctcgtggttatggcaatggtgaaacggaaaaacagc

SEQ ID NO: 22 - DNA, 57 bp, Artificial Sequence
  P2A nucleotide sequence
gccaccaacttcagcctgctgaagcaggccggcgacgtggaggagaaccccggcccc

SEQ ID NO: 23 - DNA, 813 bp, Artificial Sequence
  B13.14.1/TRAV+mCa nucleotide sequence
atggcctctgcacccatctcgatgcttgcgatgctcttcacattgagtgggctgagagctcagtcagtggctcagccggaagatcaggtcaacgttgctgaagggaatcctctgactgtgaaatgcacctattcagtctctggaaacccttatcttttttggtatgttcaataccccaaccgaggcctccagttccttctgaaatacatcacaggggataacctggttaaaggcagctatggctttgaagctgaatttaacaagagccaaacctccttccacctgaagaaaccatctgcccttgtgagcgactccgctttgtacttctgtgctgtgagagacggtaggggaggaggaaacaaactcacctttgggacaggcactcagctaaaagtggaactcgacatccagaacccagaacctgctgtgtaccagttaaaagatcctcggtctcaggacagcaccctctgcctgttcaccgactttgactcccaaatcaatgtgccgaaaaccatggaatctggaacgttcatcactgacaaaactgtgctggacatgaaagctatggattccaagagcaatggggccattgcctggagcaaccagacaagcttcacctgccaagatatcttcaaagagaccaacgccacctaccccagttcagacgttccctgtgatgccacgttgactgagaaaagctttgaaacagatatgaacctaaactttcaaaacctgtcagttatgggactccgaatcctcctgctgaaagtagccggatttaacctgctcatgacgctgaggctgtggtccagt

SEQ ID NO: 24 - DNA, 918 bp, Artificial Sequence
  B13.14.1/TRBV+mCb nucleotide sequence
atgagcaaccaggtgctctgctgtgtggtcctttgtctcctgggagcaaacaccgtggatggtggaatcactcagtccccaaagtacctgttcagaaaggaaggacagaatgtgaccctgagttgtgaacagaatttgaaccacgatgccatgtactggtaccgacaggacccagggcaagggctgagattgatctactactcacagatagtaaatgactttcagaaaggagatatagctgaagggtacagcgtctctcgggagaagaaggaatcctttcctctcactgtgacatcggcccaaaagaacccgacagctttctatctctgtgccagtagccccggacaacgagataattcacccctccactttgggaacgggaccaggctcactgtgacagaggacctgcgcaacgtcaccccaccaaaggtcagtttgtttgagccatcaaaggcggagatcgccaacaaacagaaagctacgctcgtgtgtttggctcggggcttcttcccagaccacgtagaactttcctggtgggtcaatggaaaggaggttcattccggagtgtccactgatccccaagcgtacaaggaatccaactatagctactgtctctcatctcggctccgggtgagtgcgacattctggcataatcctcggaaccactttcgatgccaagtgcagtttcatgggttgagcgaggaagacaagtggcccgagggcagtcctaaaccagtcactcaaaacataagcgccgaggcatggggtagagccgattgtgggattactagcgcttcataccaacaaggggtattgagcgctacaattctttacgaaattctcctcggcaaggcgacgctctacgccgtactggtgtctactctcgtggttatggcaatggtgaaacggaaaaacagc

SEQ ID NO: 25 - protein, 13 aa, Artificial Sequence
  TCR CDR3(alpha)General formula
  MISC_FEATURE (5)..(5): Xaa is selected from G, A, D, L, M, Q, R, S, V, W, Y
  MISC_FEATURE (6)..(6): Xaa  is selected from R, A, D, G, H, I, K, L, M, N, P, Q, S, T, V, W, Y
  MISC_FEATURE (7)..(7): Xaa is selected from G, A, D, E, F, H, I, K, L, M, N, P, Q, R, S, T, V, W, Y
AVRDXXXGGNKLT

SEQ ID NO: 26 - protein, 13 aa, Artificial Sequence
  TCR CDR3(beta)General formula
  MISC_FEATURE (4)..(4): Xaa is selected from P, A, H, M, S, T, V, Y
  MISC_FEATURE (6)..(6): Xaa is Q or S
ASSXGXRDNSPLH

SEQ ID NO: 27 - protein, 6 aa, Artificial Sequence
  TCR CDR1(alpha)General formula
  MISC_FEATURE (4)..(4): Xaa is selected from N, A, D, E, F, G, H, I, K, L, M, P, Q, R, S, T, V, W, Y
VSGXPY

SEQ ID NO: 28 - protein, 8 aa, Artificial Sequence
  TCR CDR2(alpha)General formula
  MISC_FEATURE (2)..(2): Xaa  is selected from I, A, D, E, F, G, H, K, L, M, N, P, Q, R, S, T, V, W, Y
  MISC_FEATURE (3)..(3): Xaa is selected from T, A, D, E, H, I, L, N, Q, R, S, W, Y
YXXGDNLV

SEQ ID NO: 29 - protein, 6 aa, Artificial Sequence
  TCR CDR2(beta)General formula
  MISC_FEATURE (2)..(2): Xaa is selected from Q, A, F, G, H, I, K, L, M, N, P, R, S, T, V, W, Y
  MISC_FEATURE (3)..(3): Xaa is selected from I, F, H, T, V
  MISC_FEATURE (6)..(6): Xaa is selected from D, A, E, F, G, H, I, K, L, M, N, P, Q, R, S, T, V, W, Y
SXXVNX

SEQ ID NO: 30 - protein, 45 aa, Artificial Sequence
  B13.14.1 TCR FR1(alpha)
MASAPISMLAMLFTLSGLRAQSVAQPEDQVNVAEGNPLTVKCTYS

SEQ ID NO: 31 - protein, 17 aa, Artificial Sequence
  B13.14.1 TCR FR2(alpha)
LFWYVQYPNRGLQFLLK

SEQ ID NO: 32 - protein, 34 aa, Artificial Sequence
  B13.14.1 TCR FR3(alpha)
KGSYGFEAEFNKSQTSFHLKKPSALVSDSALYFC

SEQ ID NO: 33 - protein, 11 aa, Artificial Sequence
  B13.14.1 TCR FR4(alpha)
FGTGTQLKVEL

SEQ ID NO: 34 - protein, 45 aa, Artificial Sequence
  B13.14.1 TCR FR1(beta)
MSNQVLCCVVLCLLGANTVDGGITQSPKYLFRKEGQNVTLSCEQN

SEQ ID NO: 35 - protein, 17 aa, Artificial Sequence
  B13.14.1 TCR FR2(beta)
MYWYRQDPGQGLRLIYY

SEQ ID NO: 36 - protein, 37 aa, Artificial Sequence
  B13.14.1 TCR FR3(beta)
FQKGDIAEGYSVSREKKESFPLTVTSAQKNPTAFYLC

SEQ ID NO: 37 - protein, 10 aa, Artificial Sequence
  B13.14.1 TCR FR4(beta)
FGNGTRLTVT

SEQ ID NO: 38 - protein, 17 aa, Artificial Sequence
  TCR FR2(alpha)General formula
  MISC_FEATURE (17)..(17): Xaa  is selected from K, A, D, E, F, G, H, I, L, M, N, P, Q, R, S, T, V, W, Y
LFWYVQYPNRGLQFLLX

SEQ ID NO: 39 - protein, 17 aa, Artificial Sequence
  TCR FR2(beta)General formula
  MISC_FEATURE (17)..(17): Xaa is selected from Y, A, E, F, I, K, L, M, N, P, Q, R, S, T, V, W
MYWYRQDPGQGLRLIYX

SEQ ID NO: 40 - protein, 37 aa, Artificial Sequence
  TCR FR3(beta)General formula
  MISC_FEATURE (2)..(2): Xaa is selected from Q, A, D, E, F, G, H, I, K, L, M, N, P, R, S, T, V, W, Y
FXKGDIAEGYSVSREKKESFPLTVTSAQKNPTAFYLC

SEQ ID NO: 41 - protein, 23 aa, Artificial Sequence
  G12V-T1
TEYKLVVVGAVGVGKSALTIQLI

SEQ ID NO: 42 - protein, 14 aa, Artificial Sequence
  G12V-T2
AVGVGKSALTIQLI

SEQ ID NO: 43 - protein, 11 aa, Artificial Sequence
  G12V-T4
VVVGAVGVGKS

SEQ ID NO: 44 - protein, 14 aa, Artificial Sequence
  G12V-T5
VGAVGVGKSALTIQ

SEQ ID NO: 45 - protein, 12 aa, Artificial Sequence
  G12V-T6
YKLVVVGAVGVG

SEQ ID NO: 46 - protein, 14 aa, Artificial Sequence
  G12V-T7
VVVGAVGVGKSALT

SEQ ID NO: 47 - protein, 12 aa, Artificial Sequence
  G12V-T8
LVVVGAVGVGKS

SEQ ID NO: 48 - protein, 10 aa, Artificial Sequence
  G12V-T10
YKLVVVGAVG

SEQ ID NO: 49 - protein, 9 aa, Artificial Sequence
  G12V-T11
KLVVVGAVG

SEQ ID NO: 50 - protein, 11 aa, Artificial Sequence
  G12V-T12
TEYKLVVVGAV

SEQ ID NO: 51 - protein, 10 aa, Artificial Sequence
  G12V-T13
EYKLVVVGAV

SEQ ID NO: 52 - protein, 9 aa, Artificial Sequence
  G12V-T14
YKLVVVGAV

SEQ ID NO: 53 - protein, 11 aa, Artificial Sequence
  G12V-T17
YKLVVVGAVGV

SEQ ID NO: 54 - protein, 14 aa, Artificial Sequence
  G12V-T18
TEYKLVVVGAVGVG

SEQ ID NO: 55 - protein, 15 aa, Artificial Sequence
  G12V-T19
TEYKLVVVGAVGVGK

SEQ ID NO: 56 - protein, 16 aa, Artificial Sequence
  G12V-T20
TEYKLVVVGAVGVGKS

SEQ ID NO: 57 - protein, 17 aa, Artificial Sequence
  G12V-T21
TEYKLVVVGAVGVGKSA

SEQ ID NO: 58 - protein, 13 aa, Artificial Sequence
  G12V-T15-A1
AEYKLVVVGAVGV

SEQ ID NO: 59 - protein, 13 aa, Artificial Sequence
  G12V-T15-A2
TAYKLVVVGAVGV

SEQ ID NO: 60 - protein, 13 aa, Artificial Sequence
  G12V-T15-A3
TEAKLVVVGAVGV

SEQ ID NO: 61 - protein, 13 aa, Artificial Sequence
  G12V-T15-A4
TEYALVVVGAVGV

SEQ ID NO: 62 - protein, 13 aa, Artificial Sequence
  G12V-T15-A5
TEYKAVVVGAVGV

SEQ ID NO: 63 - protein, 13 aa, Artificial Sequence
  G12V-T15-A6
TEYKLAVVGAVGV

SEQ ID NO: 64 - protein, 13 aa, Artificial Sequence
  G12V-T15-A7
TEYKLVAVGAVGV

SEQ ID NO: 65 - protein, 13 aa, Artificial Sequence
  G12V-T15-A8
TEYKLVVAGAVGV

SEQ ID NO: 66 - protein, 13 aa, Artificial Sequence
  G12V-T15-A9
TEYKLVVVAAVGV

SEQ ID NO: 67 - protein, 13 aa, Artificial Sequence
  G12V-T15-G10
TEYKLVVVAGVGV

SEQ ID NO: 68 - protein, 13 aa, Artificial Sequence
  G12V-T15-A12
TEYKLVVVGAVAV

SEQ ID NO: 69 - protein, 13 aa, Artificial Sequence
  G12V-T15-A13
TEYKLVVVGAVGA